European Patent Application EP 4 703 361 A1, published March 4, 2026. Title: PYRIDAZINONE TRPC4/5 INHIBITOR AND USE THEREOF. Applicant: SHANGHAI INSTITUTE OF MATERIA MEDICA, CHINESE ACADEMY OF SCIENCES. The sequence listing filed with the application follows.

SEQUENCE LISTING (16 sequences)

SEQ ID NO: 1 - DNA, 21 bp, synthetic construct
  source 1..21: mol_type = other DNA
tgattctacccacggcaagtt

SEQ ID NO: 2 - DNA, 21 bp, synthetic construct
  source 1..21: mol_type = other DNA
tgatgggtttcccattgatga

SEQ ID NO: 3 - DNA, 20 bp, synthetic construct
  source 1..20: mol_type = other DNA
cggagaacaagaacgtgacc

SEQ ID NO: 4 - DNA, 20 bp, synthetic construct
  source 1..20: mol_type = other DNA
attgtcttctctccgcacca

SEQ ID NO: 5 - DNA, 20 bp, synthetic construct
  source 1..20: mol_type = other DNA
gtggcttcttgtcctctcct

SEQ ID NO: 6 - DNA, 20 bp, synthetic construct
  source 1..20: mol_type = other DNA
tgtgataggtgtccaggcag

SEQ ID NO: 7 - DNA, 20 bp, synthetic construct
  source 1..20: mol_type = other DNA
catcttccaggagcgagacc

SEQ ID NO: 8 - DNA, 20 bp, synthetic construct
  source 1..20: mol_type = other DNA
gaaggggcggagatgatgac

SEQ ID NO: 9 - DNA, 20 bp, synthetic construct
  source 1..20: mol_type = other DNA
gttcagtggtgcctctgtca

SEQ ID NO: 10 - DNA, 20 bp, synthetic construct
  source 1..20: mol_type = other DNA
actgggacgacatggaaaag

SEQ ID NO: 11 - DNA, 20 bp, synthetic construct
  source 1..20: mol_type = other DNA
agcacgtctggtttggagag

SEQ ID NO: 12 - DNA, 20 bp, synthetic construct
  source 1..20: mol_type = other DNA
acattaggcgcaggaaggtc

SEQ ID NO: 13 - DNA, 22 bp, synthetic construct
  source 1..22: mol_type = other DNA
actcggacctggtcataagggc

SEQ ID NO: 14 - DNA, 22 bp, synthetic construct
  source 1..22: mol_type = other DNA
ttccgtggcaggcaagcaaagt

SEQ ID NO: 15 - DNA, 20 bp, synthetic construct
  source 1..20: mol_type = other DNA
ttgccttacgactccacctg

SEQ ID NO: 16 - DNA, 20 bp, synthetic construct
  source 1..20: mol_type = other DNA
tagatgggccctcctttggt